European Patent Application EP 4 400 173 A2, published July 17, 2024. Title: Anti-SIRPalpha antibodies. Applicant: Byondis B.V. Application EP, filed May 15, 2018. The sequence listing filed with the application follows.

SEQUENCE LISTING (40 sequences)

SEQ ID NO: 1 - protein, 117 aa, synthetic construct
  REGION 1..117: note = SEQ ID NO:1 (HC VR 1)
QSVEESGGRLVTPGTPLTLTCTVSGIDLSSYAMSWVRQAPGKGLEWIGIISSGGITYYASWAKGRFTISKTSTTVDLKIPSPTTEDTATYFCARSLWAASNYYMALWGPGTLVTVSS

SEQ ID NO: 2 - protein, 111 aa, synthetic construct
  REGION 1..111: note = SEQ ID NO:2 (LC VR 1)
AIKMTQTPASVSAAVGGTVSINCQASEDIESYLAWYQQKPGQPPKLLIYRASTLASGVSSRFKGSGSGTQFTLTISDLESADAATYYCLGDYYSSSGDTGAFGGGTEVVVK

SEQ ID NO: 3 - protein, 116 aa, synthetic construct
  REGION 1..116: note = SEQ ID NO:3 (HC VR 2)
QSVEESGGRLVTPGTPLTLTCTVSGFSLSNYAMHWVRQAPGKGLEWIGIIYTGGATSYATWAKGQFTISKTSTTVDLKITSPTTEDTATYFCARGDRDGYAYFNIWGPGTLVTVSL

SEQ ID NO: 4 - protein, 110 aa, synthetic construct
  REGION 1..110: note = SEQ ID NO:4 (LC VR 2)
QIVMTQTPFSVSAVVGGTVTIKCQASHNIGSWLAWYQQKPGQRPKLLIYDASTLASGVSSRFKGSGSGTEFTLTISGVESADAATYYCQQGYGISYVHNVFGGGTEVVVK

SEQ ID NO: 5 - protein, 116 aa, synthetic construct
  REGION 1..116: note = SEQ ID NO:5 (HC VR 3)
QSVEESGGRLVTPGTPLTLACTVSGFSLISYYISWVRQAPEKGLEYIGIINIGGGASYASWAKGRFTISKTSTTVDLKITSPTPEDTATYFCAMSYGMDTGAFNIWGPGTLVTVSL

SEQ ID NO: 6 - protein, 110 aa, synthetic construct
  REGION 1..110: note = SEQ ID NO:6 (LC VR 3)
AQVLTQTPASVSAAVGGTVTISCQSSESVYKNNFLSWYQQKPGKPPKLLIYGASTLASGVPSRFKGSGSGTQFTLTISDLESDDAATYFCQGGYRTDIYPFGGGTEVVVK

SEQ ID NO: 7 - protein, 116 aa, synthetic construct
  REGION 1..116: note = SEQ ID NO:7 (HC VR 4)
QSVEESGGRLGTPGTPLTLTCTVSGFSLSSYVMGWFRQAPGKGLEYIGIISSSGSPYYASWVNGRFTISKTSTTMDLKMNSPTTEDTATYFCARVGPLGVDYFNIWGPGTLVTVSL

SEQ ID NO: 8 - protein, 109 aa, synthetic construct
  REGION 1..109: note = SEQ ID NO:8 (LC VR 4)
DIVMTQTPSSVEAAVGGTVTIKCQAGQSINSYLAWYQQKPGQRPKLLIYYASTLESGVPSRFKGSGSGTDYTLTISDLESADAATYYCQSWHYISRSYAFGGGTEVVVK

SEQ ID NO: 9 - protein, 116 aa, synthetic construct
  REGION 1..116: note = SEQ ID NO:9 (HC VR 5)
QSVEESGGRLVTPGTPLTLTCTVSGFSLSSYVMGWFRQAAGKGLEYIGYINADGSPYYATWVNGRFTISKTPTTMDLKINSPTTEDTATYFCARVGPLGVDYFNIWGPGTLVTVSL

SEQ ID NO: 10 - protein, 109 aa, synthetic construct
  REGION 1..109: note = SEQ ID NO:10 (LC VR 5)
DIVMTQTPASVEAAVGGTVTIKCQASQSINRYLTWYQQKPGQRPKLLIYYASTLESGVPSRFEGSGSGTDYTLTISDLESADAATYYCQSYYYISRTYAFGGGTEVVVK

SEQ ID NO: 11 - protein, 116 aa, synthetic construct
  REGION 1..116: note = SEQ ID NO:11 (HC VR 6)
QSVEESGGRLVTPGTPLTLTCTVSGIDLSSYTMTWVRQAPGKGLEWIGIIYAGGSTAYASWAKGRFTISKTSTTVDLKITSPTTEDTATYFCARSSSDGYDYFNIWGPGTLVTVSL

SEQ ID NO: 12 - protein, 111 aa, synthetic construct
  REGION 1..111: note = SEQ ID NO:12 (LC VR 6)
GVVMTQTPSSVSAAVGGTVTINCQASQSIGSWLAWYQQKPGQPPKLLIYQASKLASGVPSRFSGRGSGTHFTLTISDVQSDDAATYYCQQTVTAASNVDNAFGGGTEVVVK

SEQ ID NO: 13 - protein, 115 aa, synthetic construct
  REGION 1..115: note = SEQ ID NO:13 (HC VR 7)
RSVEESGGRLVTPGTPLTLTCTVSGFSLSSHGISWVRQAPGKGLEYIGTIGTGVITYFASWAKGRFTGSKTSTTVDLKITSPTTEDTATYFCARGSAWNDPFDPWGPGTLVTVSS

SEQ ID NO: 14 - protein, 111 aa, synthetic construct
  REGION 1..111: note = SEQ ID NO:14 (LC VR 7)
ALVMTQTPASVSAAVGGTVTTKCQASQSVYGNNDLAWYQHKPGQPPKLLIYLASTLATGVPSRFSGSGSGTQFTLTITGVQSDDAATYYCLGGGDDEADNVFGGGTEVVVK

SEQ ID NO: 15 - protein, 116 aa, synthetic construct
  REGION 1..116: note = SEQ ID NO:15 (HC VR 8)
QSLEESGGRLVTPGTPLTLTCTASGVDLSNYAMGWVRQAPGKGLEWIGIIYAGGSTSYATWAKGRFTISKTSTTMDLKMTSPTTEDTATYFCARHRSDGYDYFHLWGPGTLVTVSL

SEQ ID NO: 16 - protein, 110 aa, synthetic construct
  REGION 1..110: note = SEQ ID NO:16 (LC VR 8)
AIDMTQTPASVSEPVGGTVTIKCQASQSISSWLAWYQQKPGQRPKLLIYDASKLASGVPSRFSGSGSGTEFTLTISGVQSDDAAAYYCQQGYAVSYVENIFGGGTEVVVK

SEQ ID NO: 17 - protein, 117 aa, synthetic construct
  REGION 1..117: note = SEQ ID NO:17 (HC VR 9)
QSMEESGGRLVTPGTPLTLTCTASGFSLSNYGVSWVRQAPGKGLEWIGIIYGGSDITAYASWAKGRFTISKTSTTVDLTITSPTTEDTATYFCAKSYTNGMDYYNIWGPGTLVTVSL

SEQ ID NO: 18 - protein, 108 aa, synthetic construct
  REGION 1..108: note = SEQ ID NO:18 (LC VR 9)
AFDLTQTPSSVEAPVGGTVIIKCQASQSISSYLAWYQQKPGQPPKLLIYSASTLASGVSSRFKGSGSETQFPLTISDLESADAATYYCQSYYGSRSNVFGGGTEVVVK

SEQ ID NO: 19 - protein, 129 aa, synthetic construct
  REGION 1..129: note = SEQ ID NO:19 (HC VR 29AM4-5))
EVQLVESGGGLVQPGGSLRLSCAASGFNISYYFIHWVRQAPGKGLEWVASVYSSFGYTYYADSVKGRFTISADTSKNTAYLQMNSLRAEDTAVYYCARFTFPGLFDGFFGAYLGSLDYWGQGTLVTVSS

SEQ ID NO: 20 - protein, 110 aa, synthetic construct
  REGION 1..110: note = SEQ ID NO:20 (LC VR 29AM4-5)
DIQMTQSPSSLSASVGDRVTITCRASQSVSSAVAWYQQKPGKAPKLLIYSASSLYSGVPSRFSGSRSGTDFTLTISSLQPEDFATYYCQQAVNWVGALVTFGQGTKVEIK

SEQ ID NO: 21 - protein, 121 aa, synthetic construct
  REGION 1..121: note = SEQ ID NO:21 (HC VR 12C4)
EVKLEESGGGLMQPGGSMKLSCVASGFTFSNYWMNWVRQSPEKGLEWVAEIRLKSNNYATHYAESVKGRFTISRDDSKSSVYLQMNNLRAEDTGIYYCIRDYDYDAYFDYWGQGTTLTVSS

SEQ ID NO: 22 - protein, 111 aa, synthetic construct
  REGION 1..111: note = SEQ ID NO:22 (LC VR 12C4)
DIVLTQSPASLAVSLGQRATISCRASKSVSTSGYNYMYWYQQKPGQPPKLLIYLASNLESGVPARFSGSGSGTDFTLNIHPVEEEDAATYYCQHSGELPYTFGGGTKLEIK

SEQ ID NO: 23 - protein, 113 aa, synthetic construct
  REGION 1..113: note = SEQ ID NO:23 (HC KWAR23 )
EVQLQQSGAELVKPGASVKLSCTASGFNIKDYYIHWVQQRTEQGLEWIGRIDPEDGETKYAPKFQDKATITADTSSNTAYLHLSSLTSEDTAVYYCARWGAYWGQGTLVTVSS

SEQ ID NO: 24 - protein, 108 aa, synthetic construct
  REGION 1..108: note = SEQ ID NO:24 (LC VR KWAR23)
QIVLTQSPAIMSASPGEKVTLTCSASSSVSSSYLYWYQQKPGSSPKLWIYSTSNLASGVPARFSGSGSGTSYSLTISSMEAEDAASYFCHQWSSYPRTFGAGTKLELK

SEQ ID NO: 25 - protein, 330 aa, synthetic construct [sequence omitted]

SEQ ID NO: 26 - protein, 107 aa, synthetic construct [sequence omitted]

SEQ ID NO: 27 - protein, 330 aa, synthetic construct
  REGION 1..330: note = SEQ ID NO 27: (human IgG1 antibody HC constant region LALA mutant (mutations underlined)
ASTKGPSVFPLAPSSKSTSGGTAALGCLVKDYFPEPVTVSWNSGALTSGVHTFPAVLQSSGLYSLSSVVTVPSSSLGTQTYICNVNHKPSNTKVDKKVEPKSCDKTHTCPPCPAPEAAGGPSVFLFPPKPKDTLMISRTPEVTCVVVDVSHEDPEVKFNWYVDGVEVHNAKTKPREEQYNSTYRVVSVLTVLHQDWLNGKEYKCKVSNKALPAPIEKTISKAKGQPREPQVYTLPPSRDELTKNQVSLTCLVKGFYPSDIAVEWESNGQPENNYKTTPPVLDSDGSFFLYSKLTVDKSRWQQGNVFSCSVMHEALHNHYTQKSLSLSPGK

SEQ ID NO: 28 - protein, 19 aa, synthetic construct
  REGION 1..19: note = SEQ ID NO:28 (leader sequence antibodies 1-9)
MGWSCIILFLVATATGVHS

SEQ ID NO: 29 - protein, 21 aa, synthetic construct
  REGION 1..21: note = SEQ ID NO:29 (HAVT20 leader sequence)
MACPGFLWALVISTCLEFSMA

SEQ ID NO: 30 - protein, 117 aa, synthetic construct
  REGION 1..117: note = SEQ ID NO:30 (HC10
KVEESGGGLVQPGGSLRLSCAASGFSLSSYVMGWVRQAPGKGLEWVSIISSSGSPYYASWVNGRFTISKDNSEGMVYLQMNSLRAEDTAVYYCARVGPLGVDYFNIWGQGTTVTVSS

SEQ ID NO: 31 - protein, 109 aa, synthetic construct
  REGION 1..109: note = SEQ ID NO:31 (LC 10)
DIVMTQSPDSLAVSLGERATINCQAGQSINSYLAWYQQKPGQPPKLLIYYASTLESGVPDRFSGSGSGTDFTLTISSLQAEDVAVYYCQSWHYISRSYAFGGGTKLEIK

SEQ ID NO: 32 - protein, 117 aa, synthetic construct
  REGION 1..117: note = SEQ ID NO:32 (HC VR 11)
EVKVEESGGGLVQPGGSLRLSCAASGFSLSSYVMGWVRQAPGKGLEWVSIISSSGSPYYASWVNGRFTISKTSTTMDLQMNSLRAEDTAVYYCARVGPLGVDYFNIWGQGTTVTVSS

SEQ ID NO: 33 - protein, 109 aa, synthetic construct
  REGION 1..109: note = SEQ ID NO:33 (LC VR 11)
DIQMTQSPSSLSASVGDRVTITCQAGQSINSYLAWYQQKPGKVPKLLIYYASTLESGVPSRFSGSGSGTDFTLTISSLQPEDVATYYCQSWHYISRSYAFGQGTKVEIK

SEQ ID NO: 34 - protein, 116 aa, synthetic construct
  REGION 1..116: note = SEQ ID NO:34 (HC VR 12)
VQLVESGGRLVQPGTPLTLSCTVSGFSLSSYVMGWFRQAPGKGLEYIGIISSSGSPYYASWVNGRFTISKTSTTMDLKMNSLRSEDTATYFCARVGPLGVDYFNIWGPGTLVTVSS

SEQ ID NO: 35 - protein, 115 aa, synthetic construct
  REGION 1..115: note = SEQ ID NO:35 (HC VR 13 +14)
RQLVESGGGLVQPGGSLRLSCTASGFSLSSHGISWVRQAPGKGLEYIGTIGTGVITYFASWAKGRFTGSKTSSTAYMELSSLRSEDTAVYFCARGSAWNDPFDPWGQGTLVTVSS

SEQ ID NO: 36 - protein, 111 aa, synthetic construct
  REGION 1..111: note = SEQ ID NO:36 (LC VR 13)
AIQMTQSPSSLSASVGDRVTITCQASQSVYGNNDLAWYQQKPGKAPKLLIYLASTLATGVPSRFSGSGSGTDFTLTISSLQPEDFATYYCLGGGDDEADNVFGGGTKVEIK

SEQ ID NO: 37 - protein, 111 aa, synthetic construct
  REGION 1..111: note = SEQ ID NO:37 (LC VR 14 +16)
DIEMTQSPSSVSASVGDRVTLTCQASQSVYGNNDLAWYQQKPGQAPKLLIYLASTLATGVPSRFSGSGSGTDFTLTISSLQPEDFATYYCLGGGDDEADNVFGGGTKVEIK

SEQ ID NO: 38 - protein, 111 aa, synthetic construct
  REGION 1..111: note = SEQ ID NO:38 (LC VR 15)
ELVMTQSPSSLSASVGDRVTITCQASQSVYGNNDLAWYQQKPGEAPKLLIYLASTLATGVPSRFSGSGSGTDFTLTISGLQSEDFATYYCLGGGDDEADNVFGQGTKVEIK

SEQ ID NO: 39 - protein, 19 aa, synthetic construct
  REGION 1..19: note = SEQ ID NO:39 (leader sequence heavy chains 10-14)
MGWTLVFLFLLSVTAGVHS

SEQ ID NO: 40 - protein, 20 aa, synthetic construct
  REGION 1..20: note = SEQ ID NO:40 (leader sequence light chains 10, 11, 13-16)
MVSSAQFLGLLLLCFQGTRC